European Patent Application EP 4 115 897 A1, published January 11, 2023. Title: USE OF LYSIN TO RESTORE/AUGMENT ANTIBACTERIAL ACTIVITY IN THE PRESENCE OF PULMONARY SURFACTANT OF ANTIBIOTICS INHIBITED THEREBY. Applicant: CONTRAFECT CORPORATION. Application PCT/US2016/052348. The sequence listing filed with the application follows.

SEQUENCE LISTING (16 sequences)

SEQ ID NO: 1 - DNA, 738 bp, Streptococcus suis
atgacaacagtaaatgaagcattaaataatgtaagagctcaggttgggtccggtgtgtctgttggcaacggcgaatgctacgctttggctagttggtacgagcgcatgattagtccggatgcaactgtcggacttggcgctggtgtgggctgggtcagcggtgcaatcggcgatacaatctctgccaaaaacatcggctcatcatacaactggcaagctaacggctggacagtttccacatctggtccatttaaagcaggtcagattgtgacgcttggggcaacaccaggaaacccttacggacatgtggtaatcgtcgaagcagtggacggcgatagattgactattttggagcaaaactacggcgggaaacgttatcccgtccgtaattattacagcgctgcaagctatcgtcaacaggtcgtgcattacatcacaccgcctggcacggtcgcacagtcagcacccaaccttgcaggctctcgttcctatcgcgagacgggcactatgactgtcacggtcgatgctctcaatgttcgcagggcgccaaatacttcaggcgagattgtagcagtatacaagcgtggtgaatcatttgactatgatactgtcatcatcgatgtcaatggctatgtctgggtgtcttacataggcggcagcggcaaacgtaactacgttgcgacgggcgctaccaaagacggtaagcgtttcggcaatgcttggggtacatttaaataa

SEQ ID NO: 2 - protein, 280 aa, Unknown
  source: /note="Description of Unknown: ClyS lysin sequence"
METLKQAESYIKSKVNTGTDFDGLYGYQCMDLAVDYIYHVTDGKIRMWGNAKDAINNSFGGTATVYKNYPAFRPKYGDVVVWTTGNFATYGHIAIVTNPDPYGDLQYVTVLEQNWNGNGIYKTELATIRTHDYTGITHFIRPNFATESSVKKKDTKKKPKPSNRDGINKDKIVYDRTNINYNMVLQGKSASKITVGSKAPYNLKWSKGAYFNAKIDGLGATSATRYGDNRTNYRFDVGQAVYAPGTLIYVFEIIDGWCRIYWNNHNEWIWHERLIVKEVF

SEQ ID NO: 3 - protein, 288 aa, Unknown
  source: /note="Description of Unknown: PlyV12 lysin sequence"
MTRRYTKMNVPQSLVNWFVNHRNLLTYSMYGSRNGSDGTADCSGSMSQALKEAGIPIQGLPSTVTLGQQLAKNGFYRISRNEDWNAETGDIVLMSWGADMASSGGAGGHVGVMMDSVNFISCDYSTQGAAGQAINTYPWNDYYEANKPAYIEVWRYSESAPQTKNQANTAVTPQQKAYYEANEVKYVNGIWQIKCDYLSPIGFDYLENGIPVTMVNWVDKDGNDLPDGADQDLKAGMYFSFSSDETNIVDTGNGGYYGGYYWRLFEFGQFGPVWLSCWNKDDLVNYFQ

SEQ ID NO: 4 - protein, 495 aa, Unknown
  source: /note="Description of Unknown: LysK lysin sequence"
MAKTQAEINKRLDAYAKGTVDSPYRVKKATSYDPSFGVMEAGAIDADGYYHAQCQDLITDYVLWLTDNKVRTWGNAKDQIKQSYGTGFKIHENKPSTVPKKGWIAVFTSGSYEQWGHIGIVYDGGNTSTFTILEQNWNGYANKKPTKRVDNYYGLTHFIEIPVKAGTTVKKKTAKKSASKTPAPKKKATLKVSKNHINYTMDKRGKKPEGMVIHNDAGRSSGQQYENSLANAGYARYANGIAHYYGSEGYVWEAIDAKNQIAWHTGDGTGANSGNFRFAGIEVCQSMSASDAQFLKNEQAVFQFTAEKFKEWGLTPNRKTVRLHMEFVPTACPHRSMVLHTGFNPVTQGRPSQAIMNKLKDYFIKQIKNYMDKGTSSSTVVKDGKTSSASTPATRPVTGSWKKNQYGTWYKPENATFVNGNQPIVTRIGSPFLNAPVGGNLPAGATIVYDEVCIQAGHIWIGYNAYNGNRVYCPVRTCQGVPPNQIPGVAWGVFK

SEQ ID NO: 5 - protein, 339 aa, Unknown
  source: /note="Description of Unknown: Cpl-1 lysin sequence"
MVKKNDLFVDVSSHNGYDITGILEQMGTTNTIIKISESTTYLNPCLSAQVEQSNPIGFYHFARFGGDVAEAEREAQFFLDNVPMQVKYLVLDYEDDPSGDAQANTNACLRFMQMIADAGYKPIYYSYKPFTHDNVDYQQILAQFPNSLWIAGYGLNDGTANFEYFPSMDGIRWWQYSSNPFDKNIVLLDDEEDDKPKTAGTWKQDSKGWWFRRNNGSFPYNKWEKIGGVWYYFDSKGYCLTSEWLKDNEKWYYLKDNGAMATGWVLVGSEWYYMDDSGAMVTGWVKYKNNWYYMTNERGNMVSNEFIKSGKGWYFMNTNGELADNPSFTKEPDGLITVA

SEQ ID NO: 6 - protein, 126 aa, Artificial Sequence
  source: /note="Description of Artificial Sequence: Synthetic polypeptide"
MTYTLSKRSLDNLKGVHPDLVAVVHRAIQLTPVDFAVIEGLRSVSRQKELVAAGASKTMNSRHLTGHAVDLAAYVNGIRWDWPLYDAIAVAVKAAAKELGVAIVWGGDWTTFKDGPHFELDRSKYR

SEQ ID NO: 7 - protein, 147 aa, Artificial Sequence
  source: /note="Description of Artificial Sequence: Synthetic polypeptide"
MKISLEGLSLIKKFEGCKLEAYKCSAGVWTIGYGHTAGVKEGDVCTQEEAEKLLRGDIFKFEEYVQDSVKVDLDQSQFDALVAWTFNLGPGNLRSSTMLKKLNNGEYESVPFEMRRWNKAGGKTLDGLIRRRQAESLLFESKEWHQV

SEQ ID NO: 8 - protein, 144 aa, Artificial Sequence
  source: /note="Description of Artificial Sequence: Synthetic polypeptide"
MRTSQRGIDLIKSFEGLRLSAYQDSVGVWTIGYGTTRGVTRYMTITVEQAERMLSNDIQRFEPELDRLAKVPLNQNQWDALMSFVYNLGAANLASSTLLKLLNKGDYQGAADQFPRWVNAGGKRLDGLVKRRAAERALFLEPLS

SEQ ID NO: 9 - protein, 181 aa, Artificial Sequence
  source: /note="Description of Artificial Sequence: Synthetic polypeptide"
MNNELPWVAEARKYIGLREDTSKTSHNPKLLAMLDRMGEFSNESRAWWHDDETPWCGLFVGYCLGVAGRYVVREWYRARAWEAPQLTKLDRPAYGALVTFTRSGGGHVGFIVGKDARGNLMVLGGNQSNAVSIAPFAVSRVTGYFWPSFWRNKTAVKSVPFEERYSLPLLKSNGELSTNEA

SEQ ID NO: 10 - protein, 439 aa, Artificial Sequence
  source: /note="Description of Artificial Sequence: Synthetic polypeptide"
MKRTTLNLELESNTDRLLQEKDDLLPQSVTNSSDEGTPFAQVEGASDDNTAEQDSDKPGASVADADTKPVDPEWKTITVASGDTLSTVFTKAGLSTSAMHDMLTSSKDAKRFTHLKVGQEVKLKLDPKGELQALRVKQSELETIGLDKTDKGYSFKREKAQIDLHTAYAHGRITSSLFVAGRNAGLPYNLVTSLSNIFGYDIDFALDLREGDEFDVIYEQHKVNGKQVATGNILAARFVNRGKTYTAVRYTNKQGNTSYYRADGSSMRKAFIRTPVDFARISSRFSLGRRHPILNKIRAHKGVDYAAPIGTPIKATGDGKILEAGRKGGYGNAVVIQHGQRYRTIYGHMSRFAKGIRAGTSVKQGQIIGYVGMTGLATGPHLHYEFQINGRHVDPLSAKLPMADPLGGADRKRFMAQTQPMIARMDQEKKTLLALNKQR

SEQ ID NO: 11 - protein, 39 aa, Artificial Sequence
  source: /note="Description of Artificial Sequence: Synthetic polypeptide"
NKGDYQGAADQFPRWVNAGGKRLDGLVKRRASQSRESQC

SEQ ID NO: 12 - protein, 42 aa, Artificial Sequence
  source: /note="Description of Artificial Sequence: Synthetic polypeptide"
NKGDYQGAADQFPRWVNAGGKRLDGLVKRRAAERALFLEPLS

SEQ ID NO: 13 - protein, 31 aa, Artificial Sequence
  source: /note="Description of Artificial Sequence: Synthetic polypeptide"
NKGDYQGAADQFPRWVNAGGKRLDGLVKRRA

SEQ ID NO: 14 - protein, 31 aa, Artificial Sequence
  source: /note="Description of Artificial Sequence: Synthetic polypeptide"
NKGDYQGAADQFPRWVNAGGKRLDGLVKRRK

SEQ ID NO: 15 - protein, 43 aa, Artificial Sequence
  source: /note="Description of Artificial Sequence: Synthetic polypeptide"
NKGDYQGAADQFPRWVNAGGKRLDGLVKRRAAERALFLEPLSC

SEQ ID NO: 16 - protein, 495 aa, Unknown
  Description of Unknown: PAL lysin peptide
MAKTQAEINKRLDAYAKGTVDSPYRVKKATSYDPSFGVMEAGAIDADGYYHAQCQDLITDYVLWLTDNKVRTWGNAKDQIKQSYGTGFKIHENKPSTVPKKGWIAVFTSGSYEQWGHIGIVYDGGNTSTFTILEQNWNGYANKKPTKRVDNYYGLTHFIEIPVKAGTTVKKETAKKSASKTPAPKKKATLKVSKNHINYTMDKRGKKPEGMVIHNDAGRSSGQQYENSLANAGYARYANGIAHYYGSEGYVWEAIDAKNQIAWHTGDGTGANSGNFRFAGIEVCQSMSASDAQFLKNEQAVFQFTAEKFKEWGLTPNRKTVRLHMEFVPTACPHRSMVLHTGFNPVTQGRPSQAIMNKLKDYFIKQIKNYMDKGTSSSTVVKDGKTSSASTPATRPVTGSWKKNQYGTWYKPENATFVNGNQPIVTRIGSPFLNAPVGGNLPAGATIVYDEVCIQAGHIWIGYNAYNGNRVYCPVRTCQGVPPNQIPGVAWGVFK